European Patent Application EP 4 435 118 A2, published September 25, 2024. Title: SYNTHETIC SPIKE-IN CONTROLS FOR CELL-FREE MEDIP SEQUENCING. Applicant: UNIVERSITY HEALTH NETWORK. Application EP 20884272.4, filed November 6, 2020. The sequence listing filed with the application follows.

SEQUENCE LISTING (59 sequences)

SEQ ID NO: 1 - DNA, 80 bp, synthetic construct
  misc_feature 1..80: note = Control Sequence
  source 1..80: mol_type = other DNA
tgtctaaattaaagttgtgatctttgacttagcatcgactcaccctatagcctaccagacaagaattatgaagaacatat

SEQ ID NO: 2 - DNA, 80 bp, synthetic construct
  misc_feature 1..80: note = Control Sequence
  source 1..80: mol_type = other DNA
gtacaccatcattatcctcatagcttagtctcccgcaggcccagggtacataaggcttggagattcactgttagctgctc

SEQ ID NO: 3 - DNA, 80 bp, synthetic construct
  misc_feature 1..80: note = Control Sequence
  source 1..80: mol_type = other DNA
gcctccccaactatagggtcaggaaggattatggcaccccacacgattttcacccgatctgtaccagtaatcatacatgg

SEQ ID NO: 4 - DNA, 80 bp, synthetic construct
  misc_feature 1..80: note = Control Sequence
  source 1..80: mol_type = other DNA
gctaccagtggcccccccctaccgagtcccccattaacctcacccccctgactgctaacctgggatggtgaagcctgggc

SEQ ID NO: 5 - DNA, 80 bp, synthetic construct
  misc_feature 1..80: note = Control Sequence
  source 1..80: mol_type = other DNA
ggttatgcccccgccctgcatcctccctgtctacacggcccaaccctagcaatgtgtggccccccctgctgtctcccatc

SEQ ID NO: 6 - DNA, 80 bp, synthetic construct
  misc_feature 1..80: note = Control Sequence
  source 1..80: mol_type = other DNA
gctggtgcaccgctgcccccacccacctcgcttgtcacagcctcggtaggtcctgatttgatgcttgggtgctcggctgg

SEQ ID NO: 7 - DNA, 160 bp, synthetic construct
  misc_feature 1..160: note = Control Sequence
  source 1..160: mol_type = other DNA
gtataatcataacaaaggcctaatgaaagacgctgatttgaaactagttccctcatcatctgatagatttcctcgtgtcttttttcgtgaatggcacaatatggtgtgaagacctattacaatcaaaaagtataaactagcgactaagatctcagaatta

SEQ ID NO: 8 - DNA, 80 bp, synthetic construct
  misc_feature 1..80: note = Control Sequence
  source 1..80: mol_type = other DNA
taggatataggttgtcccctagtaggagataaactttgattaacatccaattgatcgttagtgtccttcaaaattatgct

SEQ ID NO: 9 - DNA, 80 bp, synthetic construct
  misc_feature 1..80: note = Control Sequence
  source 1..80: mol_type = other DNA
tctaatactcatcttagctcgcgtgctttgtgattttagtgctgaaattcttaaatgttaaccactgtgaaatccataag

SEQ ID NO: 10 - DNA, 80 bp, synthetic construct
  misc_feature 1..80: note = Control Sequence
  source 1..80: mol_type = other DNA
ctcaaatataacaagagtagcaaacttacaaagatcgctgacaagtatgttatccatttctaagcgctaccaataacact

SEQ ID NO: 11 - DNA, 80 bp, synthetic construct
  misc_feature 1..80: note = Control Sequence
  source 1..80: mol_type = other DNA
aaggcattacttatctaatcaatcgacaaaacgttaagtcagtgttaggatagtgtcatttgtactcgtagacgaaattg

SEQ ID NO: 12 - DNA, 80 bp, synthetic construct
  misc_feature 1..80: note = Control Sequence
  source 1..80: mol_type = other DNA
ttattattgaccgtacactatttaactaacagatatgacgtattactatgatatgttaatgacgctgagctgctcggaga

SEQ ID NO: 13 - DNA, 80 bp, synthetic construct
  misc_feature 1..80: note = Control Sequence
  source 1..80: mol_type = other DNA
gaggaccatatagctcgcacaggaaccagctgaagaattgattggtagtgctgaccagacaccaaccttcaaacctctgc

SEQ ID NO: 14 - DNA, 80 bp, synthetic construct
  misc_feature 1..80: note = Control Sequence
  source 1..80: mol_type = other DNA
acaacaccctccacccaatacttgtgagttggtcgcagcacgagcctagtctccttgtaagtcagtcaaatgcctgtaac

SEQ ID NO: 15 - DNA, 80 bp, synthetic construct
  misc_feature 1..80: note = Control Sequence
  source 1..80: mol_type = other DNA
agtcatcagcatattgtcagtacccagtggtctctaggaaaatcggccggtacgtaaatactcctagtgggctgcgtggt

SEQ ID NO: 16 - DNA, 80 bp, synthetic construct
  misc_feature 1..80: note = Control Sequence
  source 1..80: mol_type = other DNA
gcttcttatgataccaaagttgcccaaaaaggctagcgttctagttagggtgcagccgcgagaagaccgggttcatgaag

SEQ ID NO: 17 - DNA, 80 bp, synthetic construct
  misc_feature 1..80: note = Control Sequence
  source 1..80: mol_type = other DNA
gcaggctgcagggtttggcccctggttccgttccagcaggtggcataggtggggaaagccaggtgcctacagtggggtgg

SEQ ID NO: 18 - DNA, 80 bp, synthetic construct
  misc_feature 1..80: note = Control Sequence
  source 1..80: mol_type = other DNA
caccttgagacctccagagggggatccacaacttgcgccctctgtgaagtaggctctggtgcgcaggggggaaggggggc

SEQ ID NO: 19 - DNA, 80 bp, synthetic construct
  misc_feature 1..80: note = Control Sequence
  source 1..80: mol_type = other DNA
ttgggaggctctggactggggcaaacgacaccgtgcatcaactgtgtggtggtggcctcgtccccccccatcctctccgc

SEQ ID NO: 20 - DNA, 160 bp, synthetic construct
  misc_feature 1..160: note = Control Sequence
  source 1..160: mol_type = other DNA
ttagtcgagattttagcctaattgagagatagtccgatgatatgtctttgatctaacatgtcatcatgaaatatgaagccaacacactcatatgttcatgtgacaaaagatccagttaagccagtattgaggtttgtccatcacttaagtactattcatt

SEQ ID NO: 21 - DNA, 160 bp, synthetic construct
  misc_feature 1..160: note = Control Sequence
  source 1..160: mol_type = other DNA
ctttactactgaatgtaagctcttgcagaggatctaacagggatagaattatgaacacgtctgtcacacataacttcaaatgcaatttattaataagggtcagaatgtgtggtatctttccagacttatatcattccctttactataaccgattacacat

SEQ ID NO: 22 - DNA, 160 bp, synthetic construct
  misc_feature 1..160: note = Control Sequence
  source 1..160: mol_type = other DNA
atgtgtaagaaataaaatactggctcatcatcataaacttgtctataatgtcactattatcacaaagaatgcaggtacgacacggtatcggcagcagtggatagctcgtatctatatgaataggggaagtgaataatatgacaatagtatactttgctta

SEQ ID NO: 23 - DNA, 160 bp, synthetic construct
  misc_feature 1..160: note = Control Sequence
  source 1..160: mol_type = other DNA
ttgtagtacagtctaaccatcttgacccagtagctccccatctgatatgctcagtagctagggtggcctgagggaaccggtcaaacccacttattctgaaccccagaggtatgttatgcgcaggaacctgccttctattggtagtgtcttgggtcaacag

SEQ ID NO: 24 - DNA, 160 bp, synthetic construct
  misc_feature 1..160: note = Control Sequence
  source 1..160: mol_type = other DNA
gtaacatggttaccactgggaccggaccttttcacctccactttcagggaataggattcagtcctgtatagcagtgtgacaccccaaggccaattccaccctacattcaatgcctgagtgtatgttggccattgggtaactagccgtgtcccaacctcat

SEQ ID NO: 25 - DNA, 160 bp, synthetic construct
  misc_feature 1..160: note = Control Sequence
  source 1..160: mol_type = other DNA
agccttggacgtgagtctctgtttctgacccaactgagatctttttactgtcattctaccccctagagactcgcgtttctagagaggggatgtatgtgaggggttgtgatttagcccgtgatgccctaggatcttgagacaattgtcagggccctccagt

SEQ ID NO: 26 - DNA, 160 bp, synthetic construct
  misc_feature 1..160: note = Control Sequence
  source 1..160: mol_type = other DNA
ggctctagggggtgataaagtctcggattatgctgtatggagtcccatcaacttccaatgacaatattgtactctaggatagctagatgacgccccaggcaaagaacccttttcgtatgaggccagccttccaaggtccactaggctcagctcctcgatg

SEQ ID NO: 27 - DNA, 160 bp, synthetic construct
  misc_feature 1..160: note = Control Sequence
  source 1..160: mol_type = other DNA
ggtaagtatgcagctcaacgagggtaccggtagcgacccgctgtttgttactagtaaggactcagtattgcgctctacttggttcctcatgacagctatgcagggatgtgttcagcccgttctaccgaacccttctaacatgagcgtgccttttgattag

SEQ ID NO: 28 - DNA, 160 bp, synthetic construct
  misc_feature 1..160: note = Control Sequence
  source 1..160: mol_type = other DNA
gcgagtaactgcttcaatgggactacaatgtgccacgggtgccctacagtcctcagccccaattgcccaaaacgaacctttcaacatcatcccggattttcactcgaagattgtgactgggggttttatgcaacaaccgagctattacatggttgcgcgt

SEQ ID NO: 29 - DNA, 160 bp, synthetic construct
  misc_feature 1..160: note = Control Sequence
  source 1..160: mol_type = other DNA
ttctcaggcagcccaccccggcagtccagatctagccccctccccttggtacttgggcatggtgagcctccgagaccccctccctctcccccctcaccagacccccccctataggtcctgcaaggtgccttcccaaacaccccagttaggcatggccacc

SEQ ID NO: 30 - DNA, 160 bp, synthetic construct
  misc_feature 1..160: note = Control Sequence
  source 1..160: mol_type = other DNA
gactcctccctaggcccccatggagccaccccctcaggccactccaggctactaggcccaggttccaggcaaatgccctctctgccagtgccactagcaacacctcccctatcaaggtggccccaggtcctcacgtagcatgcaggccccccgctccatc

SEQ ID NO: 31 - DNA, 160 bp, synthetic construct
  misc_feature 1..160: note = Control Sequence
  source 1..160: mol_type = other DNA
ccccagaggcaggtgccctaccaagctccccccatgacccctaaatcccccaccctgccccggcggttgcagtggtaccaaccagtcaggcccctcgccagtacccttccatatcttcagcctcctggccattcgatcaggagccccacagccctaggcc

SEQ ID NO: 32 - DNA, 160 bp, synthetic construct
  misc_feature 1..160: note = Control Sequence
  source 1..160: mol_type = other DNA
tagggcccgagccagcctgtaccttgcgcccctgccccccctctacctggggaccccacggtcatccttgacagggtgcccctcggcccactcccattctccttttgtctccagtaaacccccagagcccaaggtcagcctgctgcagggtttgcctcca

SEQ ID NO: 33 - DNA, 160 bp, synthetic construct
  misc_feature 1..160: note = Control Sequence
  source 1..160: mol_type = other DNA
actgctgcgcggcgcacctcccacatgtcctacccatcacctcctcagtgttcactggctgggtctgtcctcctacagggtgccaagcggggctccattgccactagaagcccatggtccagcgtggctagatccgagcggggggcctccaccagccgtc

SEQ ID NO: 34 - DNA, 160 bp, synthetic construct
  misc_feature 1..160: note = Control Sequence
  source 1..160: mol_type = other DNA
tggaggggctgggcctgctcccctagtgcggaatcctgccctccggtggcttgctctttgggtccacgggtactagaggggaattatgaccagagccctgcagccccgaagcggggtgcgccacagtccccacgactccgccaaccttcataccctgtcc

SEQ ID NO: 35 - DNA, 320 bp, synthetic construct
  misc_feature 1..320: note = Control Sequence
  source 1..320: mol_type = other DNA
aaatgtataaatttggtgaggactgtaattctagttgtactcctatgtctacaagaccatctccttactatagtgggattaataatattgtaaatccggctatgatcttagacagggaaaatgagttgtaaccgattgttaagtatcatttttccttgaattgacatcacctagcttgtcttaatgttcatgagaatttcaggctaaccacaatgtcaactatgcgacaccatgtatcatcatttccacttcacaacagaaccgggtcattttgtgtattcccatagattaaatgattaaccttatgccactataatata

SEQ ID NO: 36 - DNA, 320 bp, synthetic construct
  misc_feature 1..320: note = Control Sequence
  source 1..320: mol_type = other DNA
taatgtataaatatggtgaggactgtaattctagttgtactcctatgtctacaagaccatctccttactatagtgggattaataatattgtatatccggctatgatcttagacagggaaaatgagttgtaaccgattgttaagtatcataattccttgaattgacatcacctagcttgtcttaatgttcatgagaatttcaggctaaccacaatgtcaactatgcgacaccatgtatcatcatttccacttcacaacagaaccgggtcataatgtgtattcccatagattaaatgattaaccttatgccactataatata

SEQ ID NO: 37 - DNA, 320 bp, synthetic construct
  misc_feature 1..320: note = Control Sequence
  source 1..320: mol_type = other DNA
agcataaaaagcctataactcgattttttaacattaagcggtaccgtttctgcatccaatgacataatatatatgggagcttactattgagatgcactcttaatacggaattacgttacaaggtagagggctatgactagaattgagctttatattagcagaagtgtcttgtccagtagggtcttgaaaagttattatgtatggtgttcatgagaatcgaggtacattaaggtgaatcatttaaatcctagtatggatgttacacttcaatgcttttgtacaactaactcgggtgcgtaaatatattgaaacaatgttta

SEQ ID NO: 38 - DNA, 320 bp, synthetic construct
  misc_feature 1..320: note = Control Sequence
  source 1..320: mol_type = other DNA
actggattgtagctatgcctagcattccttctcttgagcctcaaagtcttatctgatgttcattccaacactcttgaacggattttaaaaacaaatatgtataaccgacgcaagaatttaatatatgaataagtctcctgttctagatttaatctcaatagtgattatcgaaaattagtatagatttagtgagaatagagatgtgttccttccttaatagtctttaatcttggacatggtgagcagtattatatccgactgttaagtcgagactgtctttcgtaatgtgacgccttactttttgagatagagaacctaag

SEQ ID NO: 39 - DNA, 320 bp, synthetic construct
  misc_feature 1..320: note = Control Sequence
  source 1..320: mol_type = other DNA
tactataattaggcaggtgattgaagaacctgttctttaactatcatataccagtacatacttcaactatttttgttgatcaggatctattaacgaatcacgtttgacttaatttacaacttgctcgcggtattaataaatagattttatttgccgtgttttcagtacgtataatgcgatcaagcagcaatgccggaactgttaattgtcctcgccttactgatatgtttaaacttcaacttttcgtctcgaggtttagtaaaataatgtattaaagaatacgaacgtgattatcccgacggcacactgtcacttcgtct

SEQ ID NO: 40 - DNA, 320 bp, synthetic construct
  misc_feature 1..320: note = Control Sequence
  source 1..320: mol_type = other DNA
gaacaacttatctgagaacaagactacgtcaacttttgtacgtgggataagttttcctgaattctaattataaatatggacgtgctcaatgaattaacagacgccacacgacgtttatatcggactgattacaagtttattctgtgtaagtaacaacaacgctacgatctctgtatgattgaatacagtcaaacggttctataatcactactcattctactgttcgaactaatatcaatcaagtcgttaataaatcttcatgatcactcgctatttctagaagtgactcgctaaggacgataattattcttcgttcaaaa

SEQ ID NO: 41 - DNA, 320 bp, synthetic construct
  misc_feature 1..320: note = Control Sequence
  source 1..320: mol_type = other DNA
gctaacaccatggctgctagaattaaagtattgactgactcatacgtggaatacccaagccaaccctgtcccctcaactaaaggtgattctggacctttcaagggttggcaggtatttacccctatcgacaagaagagtgacctacaggagaaatcgatcagaggcagttcaagatcaactccctggtcctcctggcctggagctcatgatgaagagtccagtgcctcctgctcaccagcatcccatgtgacgcaggtcactaggccttgtggccttaaaaagcccagcacatactgactagggcagttcagcttataca

SEQ ID NO: 42 - DNA, 320 bp, synthetic construct
  misc_feature 1..320: note = Control Sequence
  source 1..320: mol_type = other DNA
ggctcaccagtggctccccatccgatcaagctacccaactaatgtactcaaggtacataattaaggtagaaccaccgaaagtctactagtgatgttcactctgtccctgggataagagtagcataaggccactaagctccactacctcagccaacgtaatgtctctttccagcgtctgttcaaaatgctcttggtagtggttctgctaggtaagggcagttcctttgccagggtctagacctagcccagtgtggttacccccatgaacaacagggtggaggcagggtcaacccagctactggccataatttctagagtca

SEQ ID NO: 43 - DNA, 320 bp, synthetic construct
  misc_feature 1..320: note = Control Sequence
  source 1..320: mol_type = other DNA
gccactggggaccacctcattaccaggctttggcatgctgtaatgtctccgatccttgagatgccctgcccccaatcgcagatgtcagtaggcagctagcacaactgaaactactccaccccaaccgtgatcctggtgcaaggcttcccaaagaaaatatttaactaaatacagagatgctacctaaatcccgctgggagttaatcagattcgatccgcgaccccctttggtgtaagagtgtagcttgcttcttataccctctccccgctccacaataggagcctacttcaccacaccaataaggtgaacatcctatctc

SEQ ID NO: 44 - DNA, 320 bp, synthetic construct
  misc_feature 1..320: note = Control Sequence
  source 1..320: mol_type = other DNA
agggagatctagcctggctaagcaggggcaactagtgcacttctttccactccagcgcacttcaccattaatggatgtacagatgattgttagtttgactctcatcagcaattcactccctacttacgtttgtggccccttacgtctagatatggggtccgagtagcccgactgctttcctcatcagttttggcagcctgcaaccaaaccccagtagataaaggcagtgtgctacacgtccgggggtaagaagcctgggttcctttaactaagtactccaaccacattacaggggcatcccgctcagtagttgatggtca

SEQ ID NO: 45 - DNA, 320 bp, synthetic construct
  misc_feature 1..320: note = Control Sequence
  source 1..320: mol_type = other DNA
agcgggcctaggttacacccccgcaacatttctaaatgcatctagggaccttactggcacagttcagcccgccagttaattatcttattgagatcctgcagaggataatctcctttcggaattaccacaacggattcgcgtaaactagtctgcgattgctttgtaagccaagggctacactgtatccaggggctggagggtttagaagtttccgttcctcatttccgaaactagacctgataggctgtcgtgtccacggattctaccaagcattcgctccgtacccacttgctaccgactgttgccgttgcctacaggta

SEQ ID NO: 46 - DNA, 320 bp, synthetic construct
  misc_feature 1..320: note = Control Sequence
  source 1..320: mol_type = other DNA
atacctcagtttatattggacctctagctgccggttagagaaactattagaaagcacggttctatacggacattcttgggctgtatgatacaaacagaggccggtacgactacttccgctccatgtaattgacgaagagtcttctccctagagatcgcttatccttattgctaatgcttgccataggccccgcttagcacgactgccgatacgtgaatgctattgagtaccggcccagtcgtcccgcatctcccacactgaaccgggttctcagctatgtcaactgtccttcttgtctttgggtgcagggtcacctgccc

SEQ ID NO: 47 - DNA, 320 bp, synthetic construct
  misc_feature 1..320: note = Control Sequence
  source 1..320: mol_type = other DNA
tgtatgatttgaagagatttgtatatacacacattgttttgtagcatagaaaaggagtttttgtcaaccggtagcccaccctgattctcaaccaagcctgtagatctgtaattggggtcttaagtccttgttaaattctggacagcactatgattttttacattctaaatcattataccaaggtatcttgtcttatcttcagagtgtccagcctgtcgatagatcggaatacaatcgtataattaattgttaagcatgtttcttgtacatacaggtcagttacatcaacatacttataaacagtgctgtaatatttgtga

SEQ ID NO: 48 - DNA, 320 bp, synthetic construct
  misc_feature 1..320: note = Control Sequence
  source 1..320: mol_type = other DNA
gcaattgatgataactgtgagtgattttgtttcttttggagactacctaacgcttatgactttgagtttctggtatgattcaaaagtagaatacctgtagcacgagcaccaatatcattgttaactgaggaagttcatgtacttaccgaattataggaaaattcagtagcttttctttgcctactaacttaggttgtgttcatcgaaatcataacatcacataactattgtcttccataagcactcaggacttcaagtaaaaaggatgaagcctattccatttcacatctgaataactttagcaaagtgtaagaagctaa

SEQ ID NO: 49 - DNA, 320 bp, synthetic construct
  misc_feature 1..320: note = Control Sequence
  source 1..320: mol_type = other DNA
cccatgcatcaaactggctccctcgtcttccgattgtctagctcataggctctcgaagcatctaagggctattccgggtcctgcaagtataagcttcattattcctaaggatgtggggagtgactcagaggtccagatcgcactgtgggccagactgacacagcttcaaaggaagggcctccaagtccactgcactcagaattaagaattccctgacgcattatcttgagaaaggcactggtccatgtctcttgtatctccgagaccaacttaaaggagggatgggagctaacaggcacctcccgacttatcttaccagt

SEQ ID NO: 50 - DNA, 320 bp, synthetic construct
  misc_feature 1..320: note = Control Sequence
  source 1..320: mol_type = other DNA
gaacttccaaatacaccgtcccatctgttcagtcagggattggggtgagagatatatcgcatcaggaattacgaaaccttatgggcaagcagtgattagctaagcctggaaacctggcaattaacacctcaaactggatccatgcctttctaactatttcccaccccttggcagtctagggctggcgagaggccctgctaatacttgaggcgtagatggggggcggcttctctgcaaactggtgcccgctggggctctaataattattcttccttgttccacacaaccagcccctcgactttaagcagctatgctatgca

SEQ ID NO: 51 - DNA, 320 bp, synthetic construct
  misc_feature 1..320: note = Control Sequence
  source 1..320: mol_type = other DNA
ttcggcacttgtctgccctcgtcagaaaatgttgggtaaaaccctaggttgtagtttgggtctggcgagcgggaaagtgcatgctcggcccatgtgggctccaaactgaaggttattagattcctagatggtgagaccgcatacaaaaagggccctggaaagaggtcacttcaacgcatctcctgatattggtctggtatccacagtagagctattgtcgcctaacagtgatgccgcgccgtcctgtattggtgcgcgagacagcttatacgtacctgaatggcgataattatccgaggggcagactcaagcttaagaaa

SEQ ID NO: 52 - DNA, 320 bp, synthetic construct
  misc_feature 1..320: note = Control Sequence
  source 1..320: mol_type = other DNA
ttgggccgccttgtccgcaaccagcaaccgatagcagtcggactccgagtcagtagtgaagtgctttagcgttaagtgtttattgtgaatgagccctctctcccccaaatcacaagaggtggcggaaaaacacgaagccgaagtacaccgacaaggaacggtgctctcaagagttgccagccattgctagacagagtaatttcctcctccaggcggaattcaacagtcctcagtcccagaattatcttgggaaaggatggacacgaatatttggaacagtggacgccgacccgtttaattacagggttccctgagattgt

SEQ ID NO: 53 - DNA, 80 bp, synthetic construct
  misc_feature 1..80: note = Control Sequence
  source 1..80: mol_type = other DNA
tgtctaaattaaagttgtgatctttgacttagcaacgtctcaccctatagcctaccagacaagaattatgaagaacatat

SEQ ID NO: 54 - DNA, 80 bp, synthetic construct
  misc_feature 1..80: note = Control Sequence
  source 1..80: mol_type = other DNA
gtacaccatcattatcctcatagcttaggctccacgtgcctacagggccataaggcttggagattcactgttagctgctc

SEQ ID NO: 55 - DNA, 80 bp, synthetic construct
  misc_feature 1..80: note = Control Sequence
  source 1..80: mol_type = other DNA
gcctccccaactatagggtcaggaaggattatggcaccccacacgtatttcacccgatctgtaccagtaatcatacatgg

SEQ ID NO: 56 - DNA, 80 bp, synthetic construct
  misc_feature 1..80: note = Control Sequence
  source 1..80: mol_type = other DNA
gctaccagtggcccccccctaccggatccatccctaacctcacccccctgactgctaacctgggatggtgaagcctgggc

SEQ ID NO: 57 - DNA, 80 bp, synthetic construct
  misc_feature 1..80: note = Control Sequence
  source 1..80: mol_type = other DNA
ggttatgcccccgccctgcatcctccctgtcacacgtgcccaaccctagcaatgtgtggccccccctgctgtctcccatc

SEQ ID NO: 58 - DNA, 80 bp, synthetic construct
  misc_feature 1..80: note = Control Sequence
  source 1..80: mol_type = other DNA
gctggtgcaccgctgcccccaccctccacgtctgtcacagcctcggtaggtcctgatttgatgcttgggtgctcggctgg

SEQ ID NO: 59 - DNA, 160 bp, synthetic construct
  misc_feature 1..160: note = Control Sequence
  source 1..160: mol_type = other DNA
gtataatcataacaaaggcctaatgaaagacgctgatttgaacatagttccctcatcatctgatattgtcctacgtgtcttttttcgatgagtgcacaatatggtgtgaagacctattacaatcaaaaagtataaactagcgactaagatctcagaatta